European Patent Application EP 4 410 817 A1, published August 7, 2024. Title: PEPTIDE HAVING ANTI-AGING ACTIVITY, AND USE THEREOF. Applicant: CAREGEN CO., LTD. Application KR. The sequence listing filed with the application follows.

SEQUENCE LISTING (13 sequences)

SEQ ID NO: 1 - protein, 12 aa, synthetic construct
DSSPLRSPSYAS

SEQ ID NO: 2 - DNA, 20 bp, synthetic construct
  source 1..20: mol_type = other DNA
caccctcaagagcctgagtc

SEQ ID NO: 3 - DNA, 20 bp, synthetic construct
  source 1..20: mol_type = other DNA
agacggctgagtagggaaca

SEQ ID NO: 4 - DNA, 20 bp, synthetic construct
  source 1..20: mol_type = other DNA
ccaggaaccgagtacaccat

SEQ ID NO: 5 - DNA, 20 bp, synthetic construct
  source 1..20: mol_type = other DNA
atacccaggttgggtgatga

SEQ ID NO: 6 - DNA, 20 bp, synthetic construct
  source 1..20: mol_type = other DNA
gcaagacctggctttggact

SEQ ID NO: 7 - DNA, 21 bp, synthetic construct
  source 1..21: mol_type = other DNA
gggagtttctggttagggctg

SEQ ID NO: 8 - DNA, 19 bp, synthetic construct
  source 1..19: mol_type = other DNA
tcagtggctggaacagtga

SEQ ID NO: 9 - DNA, 20 bp, synthetic construct
  source 1..20: mol_type = other DNA
tctggcatgtcccactatca

SEQ ID NO: 10 - DNA, 20 bp, synthetic construct
  source 1..20: mol_type = other DNA
ccttcttgggtgctggaata

SEQ ID NO: 11 - DNA, 20 bp, synthetic construct
  source 1..20: mol_type = other DNA
acacgataagggaggctgtg

SEQ ID NO: 12 - DNA, 20 bp, synthetic construct
  source 1..20: mol_type = other DNA
ggagccaaaagggtcatcat

SEQ ID NO: 13 - DNA, 20 bp, synthetic construct
  source 1..20: mol_type = other DNA
gtgatggcatggactgtggt